European Patent Application EP 4 800 076 A1, published September 2, 2026. Title: 組成物. Applicant: 国立大学法人東海国立大学機構. The sequence listing filed with the application follows.

SEQUENCE LISTING (22 sequences)

SEQ ID NO: 1 - skipped

SEQ ID NO: 2 - protein, 5 aa, synthetic construct
  REGION 1..5: note = P block
  SITE 4: note = MISC_FEATURE - X may be any amino acid
VPGXG

SEQ ID NO: 3 - protein, 5 aa, synthetic construct
  REGION 1..5: note = G block
VGGVG

SEQ ID NO: 4 - protein, 5 aa, synthetic construct
  REGION 1..5: note = P block
  SITE 4: note = MISC_FEATURE - X is Val or Phe
VPGXG

SEQ ID NO: 5 - protein, 196 aa, synthetic construct
  REGION 1..196: note = GPG1
MKLVGGVGVGGVGVGGVGVGGVGVGGVGLWLGSGVPGVGVPGVGVPGFGVPGVGVPGVGVPGVGVPGVGVPGFGVPGVGVPGVGVPGVGVPGVGVPGFGVPGVGVPGVGVPGVGVPGVGVPGFGVPGVGVPGVGVPGVGVPGVGVPGFGVPGVGVPGVGKLVGGVGVGGVGVGGVGVGGVGVGGVGLWLEHHHHHH

SEQ ID NO: 6 - protein, 205 aa, synthetic construct
  REGION 1..205: note = GPG3
MKLVGGVGVGGVGVGGVGVGGVGVGGVGLWLGSGVPGVGVPGVGVPGFGVPGVGVPGVGVPGVGVPGVGVPGFGVPGVGVPGVGVPGVGVPGVGVPGFGVPGVGVPGVGVPGVGVPGVGVPGFGVPGVGVPGVGVPGVGVPGVGVPGFGVPGVGVPGVGKLVGGVGVGGVGVGGVGVGGVGVGGVGLWLEHHHHHHKAAKGRGDS

SEQ ID NO: 7 - protein, 6 aa, synthetic construct
  REGION 1..6: note = Linker 1
LWLGSG

SEQ ID NO: 8 - protein, 4 aa, synthetic construct
KAAK

SEQ ID NO: 9 - protein, 5 aa, synthetic construct
GRGDS

SEQ ID NO: 10 - protein, 4 aa, synthetic construct
  REGION 1..4: note = RGDS
RGDS

SEQ ID NO: 11 - protein, 8 aa, synthetic construct
  REGION 1..8: note = LPGFPGLK
LPGFPGLK

SEQ ID NO: 12 - protein, 8 aa, synthetic construct
  REGION 1..8: note = LPGFPGTP
LPGFPGTP

SEQ ID NO: 13 - protein, 9 aa, synthetic construct
  REGION 1..9: note = GPPGLSGPP
GPPGLSGPP

SEQ ID NO: 14 - protein, 8 aa, synthetic construct
  REGION 1..8: note = FPGPPGPP
FPGPPGPP

SEQ ID NO: 15 - protein, 8 aa, synthetic construct
  REGION 1..8: note = LPGLPGPP
LPGLPGPP

SEQ ID NO: 16 - protein, 8 aa, synthetic construct
  REGION 1..8: note = FPGLPGPP
FPGLPGPP

SEQ ID NO: 17 - protein, 10 aa, synthetic construct
  REGION 1..10: note = GPPGPPGSPG
GPPGPPGSPG

SEQ ID NO: 18 - protein, 8 aa, synthetic construct
  REGION 1..8: note = LPGPPGPP
LPGPPGPP

SEQ ID NO: 19 - protein, 9 aa, synthetic construct
  REGION 1..9: note = FPGSPGFPG
FPGSPGFPG

SEQ ID NO: 20 - protein, 9 aa, synthetic construct
  REGION 1..9: note = GSPGLPGTP
GSPGLPGTP

SEQ ID NO: 21 - protein, 8 aa, synthetic construct
  REGION 1..8: note = IGLSGEKG
IGLSGEKG

SEQ ID NO: 22 - protein, 4 aa, synthetic construct
  REGION 1..4: note = REDV
REDV